European Patent Application EP 4 548 758 A1, published May 7, 2025. Title: 用于制备抗体的基因修饰小鼠及其制备方法. Applicant: 赛业（苏州）生物科技有限公司. The sequence listing filed with the application follows.

SEQUENCE LISTING (93 sequences)

SEQ ID NO: 1 - DNA, 21 bp, synthetic construct
  source 1..21: mol_type = other DNA
gcccatttgaaggagaggtcg

SEQ ID NO: 2 - DNA, 25 bp, synthetic construct
  source 1..25: mol_type = other DNA
catctcagctcagaacagtccagtg

SEQ ID NO: 3 - DNA, 21 bp, synthetic construct
  source 1..21: mol_type = other DNA
acaggcagggaacagaatgtg

SEQ ID NO: 4 - DNA, 21 bp, synthetic construct
  source 1..21: mol_type = other DNA
tgggctatgaactaatgaccc

SEQ ID NO: 5 - DNA, 22 bp, synthetic construct
  source 1..22: mol_type = other DNA
gcatcgcattgtctgagtaggt

SEQ ID NO: 6 - DNA, 20 bp, synthetic construct
  source 1..20: mol_type = other DNA
gatggagctgaggtctgtgc

SEQ ID NO: 7 - DNA, 20 bp, synthetic construct
  source 1..20: mol_type = other DNA
tctcaccagccacattcaag

SEQ ID NO: 8 - DNA, 22 bp, synthetic construct
  source 1..22: mol_type = other DNA
gacaccatttcacctctgttga

SEQ ID NO: 9 - DNA, 22 bp, synthetic construct
  source 1..22: mol_type = other DNA
gaatggacaaccaatgactggc

SEQ ID NO: 10 - DNA, 22 bp, synthetic construct
  source 1..22: mol_type = other DNA
cgtgctacttccatttgtcacg

SEQ ID NO: 11 - DNA, 21 bp, synthetic construct
  source 1..21: mol_type = other DNA
gccttctagttgccagccatc

SEQ ID NO: 12 - DNA, 21 bp, synthetic construct
  source 1..21: mol_type = other DNA
ccagcctacagccatagagcc

SEQ ID NO: 13 - DNA, 20 bp, synthetic construct
  source 1..20: mol_type = other DNA
ccagagccaactccaggagc

SEQ ID NO: 14 - DNA, 22 bp, synthetic construct
  source 1..22: mol_type = other DNA
gccaccagccagtagttcttcc

SEQ ID NO: 15 - DNA, 22 bp, synthetic construct
  source 1..22: mol_type = other DNA
cagagccagtgcagacagaggc

SEQ ID NO: 16 - DNA, 23 bp, synthetic construct
  source 1..23: mol_type = other DNA
ctgtccctctgtctggtgtctgg

SEQ ID NO: 17 - DNA, 20 bp, synthetic construct
  source 1..20: mol_type = other DNA
agcggaacacccacagagac

SEQ ID NO: 18 - DNA, 21 bp, synthetic construct
  source 1..21: mol_type = other DNA
atctgaggccgcacctgacac

SEQ ID NO: 19 - DNA, 22 bp, synthetic construct
  source 1..22: mol_type = other DNA
cggaacacccacagagaccgag

SEQ ID NO: 20 - DNA, 24 bp, synthetic construct
  source 1..24: mol_type = other DNA
ggcatttctcactgtcacttctgg

SEQ ID NO: 21 - DNA, 22 bp, synthetic construct
  source 1..22: mol_type = other DNA
ctccttcatggctcttagctcc

SEQ ID NO: 22 - DNA, 21 bp, synthetic construct
  source 1..21: mol_type = other DNA
aggtcagcattctggtccagg

SEQ ID NO: 23 - DNA, 25 bp, synthetic construct
  source 1..25: mol_type = other DNA
cctgagagaatgatgtgctgagacc

SEQ ID NO: 24 - DNA, 22 bp, synthetic construct
  source 1..22: mol_type = other DNA
ggaatgagggttgggtgtccaa

SEQ ID NO: 25 - DNA, 22 bp, synthetic construct
  source 1..22: mol_type = other DNA
ggactcagcagtaaccctcagg

SEQ ID NO: 26 - DNA, 22 bp, synthetic construct
  source 1..22: mol_type = other DNA
gatgatgggatagggactttgg

SEQ ID NO: 27 - DNA, 22 bp, synthetic construct
  source 1..22: mol_type = other DNA
gtgataataagcggatgaatgg

SEQ ID NO: 28 - DNA, 21 bp, synthetic construct
  source 1..21: mol_type = other DNA
gtggattgctgctgtgtcctg

SEQ ID NO: 29 - DNA, 25 bp, synthetic construct
  source 1..25: mol_type = other DNA
ctcttgttctgtaattcctccttcc

SEQ ID NO: 30 - DNA, 22 bp, synthetic construct
  source 1..22: mol_type = other DNA
caagatggagtctgcctgcttc

SEQ ID NO: 31 - DNA, 21 bp, synthetic construct
  source 1..21: mol_type = other DNA
agacgtggtgaaccgagctgt

SEQ ID NO: 32 - DNA, 23 bp, synthetic construct
  source 1..23: mol_type = other DNA
ccgtgtattactttgagggacac

SEQ ID NO: 33 - DNA, 20 bp, synthetic construct
  source 1..20: mol_type = other DNA
cctcatagtgtcctgagcgc

SEQ ID NO: 34 - DNA, 26 bp, synthetic construct
  source 1..26: mol_type = other DNA
ccttacccacactatctcttgtgtcc

SEQ ID NO: 35 - DNA, 23 bp, synthetic construct
  source 1..23: mol_type = other DNA
caggctcccaggtgctctaattc

SEQ ID NO: 36 - DNA, 22 bp, synthetic construct
  source 1..22: mol_type = other DNA
ctggacgagcagaacgtgatcg

SEQ ID NO: 37 - DNA, 25 bp, synthetic construct
  source 1..25: mol_type = other DNA
cgaagaaggcgtagatctcgtcctc

SEQ ID NO: 38 - DNA, 22 bp, synthetic construct
  source 1..22: mol_type = other DNA
ccatatcttgctccttcatggc

SEQ ID NO: 39 - DNA, 21 bp, synthetic construct
  source 1..21: mol_type = other DNA
gcaggctccaccagacctctc

SEQ ID NO: 40 - DNA, 22 bp, synthetic construct
  source 1..22: mol_type = other DNA
gtaggcgtgtacggtgggaggt

SEQ ID NO: 41 - DNA, 23 bp, synthetic construct
  source 1..23: mol_type = other DNA
tccaggtatgctcagaaaacgcc

SEQ ID NO: 42 - DNA, 22 bp, synthetic construct
  source 1..22: mol_type = other DNA
gactcagcaaacgcttctctgg

SEQ ID NO: 43 - DNA, 22 bp, synthetic construct
  source 1..22: mol_type = other DNA
tctcaactccatcgtgacggtg

SEQ ID NO: 44 - DNA, 24 bp, synthetic construct
  source 1..24: mol_type = other DNA
gcaccaccttcttgtcagttcagc

SEQ ID NO: 45 - DNA, 21 bp, synthetic construct
  source 1..21: mol_type = other DNA
gacaggtcccaggagcaggtg

SEQ ID NO: 46 - DNA, 25 bp, synthetic construct
  source 1..25: mol_type = other DNA
aatggaaagtccctattggcgttac

SEQ ID NO: 47 - DNA, 22 bp, synthetic construct
  source 1..22: mol_type = other DNA
tgcatcgcattgtctgagtagg

SEQ ID NO: 48 - DNA, 21 bp, synthetic construct
  source 1..21: mol_type = other DNA
ttgagaccgaggctagatgcc

SEQ ID NO: 49 - DNA, 20 bp, synthetic construct
  source 1..20: mol_type = other DNA
cataccgacgatctgcgacc

SEQ ID NO: 50 - DNA, 22 bp, synthetic construct
  source 1..22: mol_type = other DNA
ctggagccttatgaggttgcac

SEQ ID NO: 51 - DNA, 20 bp, synthetic construct
  source 1..20: mol_type = other DNA
ggcctgatccaaagagaggc

SEQ ID NO: 52 - DNA, 22 bp, synthetic construct
  source 1..22: mol_type = other DNA
cagggaggaatctgggaccatc

SEQ ID NO: 53 - DNA, 25 bp, synthetic construct
  source 1..25: mol_type = other DNA
aatgctggttacttgtgcttgaatt

SEQ ID NO: 54 - DNA, 23 bp, synthetic construct
  source 1..23: mol_type = other DNA
agaaggtgggagcatgatgagtc

SEQ ID NO: 55 - DNA, 21 bp, synthetic construct
  source 1..21: mol_type = other DNA
gccagaggccacttgtgtagc

SEQ ID NO: 56 - DNA, 23 bp, synthetic construct
  source 1..23: mol_type = other DNA
agaaggtgggagcatgatgagtc

SEQ ID NO: 57 - DNA, 20 bp, synthetic construct
  source 1..20: mol_type = other DNA
tggtgtctctttgcgggctt

SEQ ID NO: 58 - DNA, 23 bp, synthetic construct
  source 1..23: mol_type = other DNA
tggttgctacgcctgaataagtg

SEQ ID NO: 59 - DNA, 20 bp, synthetic construct
  source 1..20: mol_type = other DNA
atgcaagtgtgtcgctgtcg

SEQ ID NO: 60 - DNA, 24 bp, synthetic construct
  source 1..24: mol_type = other DNA
ggtgtgtcaagttgtcctctccat

SEQ ID NO: 61 - DNA, 22 bp, synthetic construct
  source 1..22: mol_type = other DNA
catggtggtgcttgaggattgc

SEQ ID NO: 62 - DNA, 24 bp, synthetic construct
  source 1..24: mol_type = other DNA
gagagcattgatgaacactgatgg

SEQ ID NO: 63 - DNA, 21 bp, synthetic construct
  source 1..21: mol_type = other DNA
gggcctgggtagggaagtgtt

SEQ ID NO: 64 - DNA, 22 bp, synthetic construct
  source 1..22: mol_type = other DNA
ccactggcagcagtgagatgag

SEQ ID NO: 65 - DNA, 24 bp, synthetic construct
  source 1..24: mol_type = other DNA
tgcaccaggaactcaaggaagatc

SEQ ID NO: 66 - DNA, 21 bp, synthetic construct
  source 1..21: mol_type = other DNA
catccagcctgcttgaactcc

SEQ ID NO: 67 - DNA, 23 bp, synthetic construct
  source 1..23: mol_type = other DNA
gtgtgatggtgttggtggagtcc

SEQ ID NO: 68 - DNA, 21 bp, synthetic construct
  source 1..21: mol_type = other DNA
gagcaggttcaaggctcaacc

SEQ ID NO: 69 - DNA, 26 bp, synthetic construct
  source 1..26: mol_type = other DNA
gagaggaatccataacttcgtatagc

SEQ ID NO: 70 - DNA, 22 bp, synthetic construct
  source 1..22: mol_type = other DNA
acaaatatccacatagaagcaa

SEQ ID NO: 71 - DNA, 23 bp, synthetic construct
  source 1..23: mol_type = other DNA
tcaggacatagcgttggctaccc

SEQ ID NO: 72 - DNA, 24 bp, synthetic construct
  source 1..24: mol_type = other DNA
agtgaccactgtgggcacagggga

SEQ ID NO: 73 - DNA, 20 bp, synthetic construct
  source 1..20: mol_type = other DNA
ggtgagaattctttgttcag

SEQ ID NO: 74 - DNA, 22 bp, synthetic construct
  source 1..22: mol_type = other DNA
aggtgcctggggaatcactcag

SEQ ID NO: 75 - DNA, 21 bp, synthetic construct
  source 1..21: mol_type = other DNA
tgtgccttctagttgccagcc

SEQ ID NO: 76 - DNA, 21 bp, synthetic construct
  source 1..21: mol_type = other DNA
gtggaatgtgtgcgaggccag

SEQ ID NO: 77 - DNA, 23 bp, synthetic construct
  source 1..23: mol_type = other DNA
tatgatgttagctatgaacttgt

SEQ ID NO: 78 - DNA, 22 bp, synthetic construct
  source 1..22: mol_type = other DNA
gtctgagccctgtgttgacagt

SEQ ID NO: 79 - DNA, 19 bp, synthetic construct
  source 1..19: mol_type = other DNA
accctggaaggtgccactc

SEQ ID NO: 80 - DNA, 22 bp, synthetic construct
  source 1..22: mol_type = other DNA
gacttctcttggtcccagtcca

SEQ ID NO: 81 - DNA, 22 bp, synthetic construct
  source 1..22: mol_type = other DNA
cacaactggcagttatcatgta

SEQ ID NO: 82 - DNA, 21 bp, synthetic construct
  source 1..21: mol_type = other DNA
gcctctcggcctgtcaagcag

SEQ ID NO: 83 - DNA, 21 bp, synthetic construct
  source 1..21: mol_type = other DNA
cagactggtgccaggaaagca

SEQ ID NO: 84 - DNA, 21 bp, synthetic construct
  source 1..21: mol_type = other DNA
agtgctcacacagctctgccc

SEQ ID NO: 85 - DNA, 22 bp, synthetic construct
  source 1..22: mol_type = other DNA
ggtgtctgttacttttgcagaa

SEQ ID NO: 86 - DNA, 21 bp, synthetic construct
  source 1..21: mol_type = other DNA
agtgctcacacagctctgccc

SEQ ID NO: 87 - DNA, 22 bp, synthetic construct
  source 1..22: mol_type = other DNA
ggtgtctgttacttttgcagaa

SEQ ID NO: 88 - DNA, 22 bp, synthetic construct
  source 1..22: mol_type = other DNA
ggatgctgccacattcccacct

SEQ ID NO: 89 - DNA, 22 bp, synthetic construct
  source 1..22: mol_type = other DNA
aagccatgtgaggcaggatcct

SEQ ID NO: 90 - DNA, 22 bp, synthetic construct
  source 1..22: mol_type = other DNA
cttgtcagtgaggaagtccccc

SEQ ID NO: 91 - DNA, 22 bp, synthetic construct
  source 1..22: mol_type = other DNA
tagcactgtggtagctactacc

SEQ ID NO: 92 - DNA, 22 bp, synthetic construct
  source 1..22: mol_type = other DNA
tgggcacagctcgggctaccac

SEQ ID NO: 93 - DNA, 22 bp, synthetic construct
  source 1..22: mol_type = other DNA
ggtgtctgttacttttgcagaa